European Patent Application EP 4 306 132 A1, published January 17, 2024. Title: Composition for delivering RNA and Preparing method for the same. Applicant: EYEGENE INC. The sequence listing filed with the application follows.

SEQUENCE LISTING (3 sequences)

SEQ ID NO: 1 - RNA, 936 nt, Artificial Sequence
  Renilla mRNA
augaccagcaagguguacgaccccgagcagcggaagcggaugaucaccggcccccaguggugggcccggugcaagcagaugaacgugcuggacagcuucaucaacuacuacgacagcgagaagcacgccgagaacgccgugaucuuccugcacggcaacgccgccagcagcuaccuguggcggcacguggugccccacaucgagcccguggcccggugcaucauccccgaccugaucggcaugggcaagagcggcaagagcggcaacggcagcuaccggcugcuggaccacuacaaguaccugaccgccugguucgagcugcugaaccugcccaagaagaucaucuucgugggccacgacuggggcgccugccuggccuuccacuacagcuacgagcaccaggacaagaucaaggccaucgugcacgccgagagcgugguggacgugaucgagagcugggacgaguggcccgacaucgaggaggacaucgcccugaucaagagcgaggagggcgagaagauggugcuggagaacaacuucuucguggagaccaugcugcccagcaagaucaugcggaagcuggagcccgaggaguucgccgccuaccuggagcccuucaaggagaagggcgaggugcggcggcccacccugagcuggccccgggagaucccccuggugaagggcggcaagcccgacguggugcagaucgugcggaacuacaacgccuaccugcgggccagcgacgaccugcccaagauguucaucgagagcgaccccggcuucuucagcaacgccaucguggagggcgccaagaaguuccccaacaccgaguucgugaaggugaagggccugcacuucagccaggaggacgcccccgacgagaugggcaaguacaucaagagcuucguggagcgggugcugaagaacgagcaguga

SEQ ID NO: 2 - RNA, 720 nt, Artificial Sequence
  EGFP mRNA
auggugagcaagggcgaggagcuguucaccgggguggugcccauccuggucgagcuggacggcgacguaaacggccacaaguucagcguguccggcgagggcgagggcgaugccaccuacggcaagcugacccugaaguucaucugcaccaccggcaagcugcccgugcccuggcccacccucgugaccacccugaccuacggcgugcagugcuucagccgcuaccccgaccacaugaagcagcacgacuucuucaaguccgccaugcccgaaggcuacguccaggagcgcaccaucuucuucaaggacgacggcaacuacaagacccgcgccgaggugaaguucgagggcgacacccuggugaaccgcaucgagcugaagggcaucgacuucaaggaggacggcaacauccuggggcacaagcuggaguacaacuacaacagccacaacgucuauaucauggccgacaagcagaagaacggcaucaaggugaacuucaagauccgccacaacaucgaggacggcagcgugcagcucgccgaccacuaccagcagaacacccccaucggcgacggccccgugcugcugcccgacaaccacuaccugagcacccaguccgcccugagcaaagaccccaacgagaagcgcgaucacaugguccugcuggaguucgugaccgccgccgggaucacucucggcauggacgagcuguacaaguaa

SEQ ID NO: 3 - RNA, 3822 nt, Artificial Sequence
  CoV2-F004 mRNA
auguucguguuccuggugcugcugccucugguguccagccagugugugaaccugaccaccagaacacagcugccuccagccuacaccaacagcuuuaccagaggcguguacuaccccgacaagguguucagauccagcgugcugcacucuacccaggaccuguuccugccuuucuucagcaacgugaccugguuccacgccauccacguguccggcaccaauggcaccaagagauucgacaaccccgugcugcccuucaacgacgggguguacuuugccagcaccgagaaguccaacaucaucagaggcuggaucuucggcaccacacuggacagcaagacccagagccugcugaucgugaacaacgccaccaacguggucaucaaagugugcgaguuccaguucugcaacgaccccuuccugggcgucuacuaccacaagaacaacaagagcuggauggaaagcgaguuccggguguacagcagcgccaacaacugcaccuucgaguacgugucccagccuuuccugauggaccuggaaggcaagcagggcaacuucaagaaccugcgcgaguucguguuuaagaacaucgacggcuacuucaagaucuacagcaagcacaccccuaucaaccucgugcgggaucugccucagggcuucucugcucuggaaccccugguggaucugcccaucggcaucaacaucacccgguuucagacacugcuggcccugcacagaagcuaccugacaccuggcgauagcagcagcggauggacagcuggugccgccgcuuacuaugugggcuaccugcagccuagaaccuuccugcugaaguacaacgagaacggcaccaucaccgacgccguggauugugcucuggauccucugagcgagacaaagugcacccugaaguccuucaccguggaaaagggcaucuaccagaccagcaacuuccgggugcagcccaccgaauccaucgugcgguuccccaauaucaccaaucugugccccuucggcgagguguucaaugccaccagauucgccucuguguacgccuggaaccggaagcggaucagcaauugcguggccgacuacuccgugcuguacaacuccgccagcuucagcaccuucaagugcuacggcguguccccuaccaagcugaacgaccugugcuucacaaacguguacgccgacagcuucgugauccggggagaugaagugcggcagauugccccuggacagacaggcaagaucgccgacuacaacuacaagcugcccgacgacuucaccggcugugugauugccuggaacagcaacaaccuggacuccaaagucggcggcaacuacaauuaccuguaccggcuguuccggaaguccaaucugaagcccuucgagcgggacaucuccaccgagaucuaucaggccggcagcaccccuuguaacggcguggaaggcuucaacugcuacuucccacugcaguccuacggcuuucagcccacaaauggcgugggcuaucagcccuacagagugguggugcugagcuucgaacugcugcaugccccugccacagugugcggcccuaagaaaagcaccaaucucgugaagaacaaaugcgugaacuucaacuucaacggccugaccggcaccggcgugcugacagagagcaacaagaaguuccugccauuccagcaguuuggccgggauaucgccgauaccacagacgccguuagagauccccagacacuggaaauccuggacaucaccccuugcagcuucggcggagugucugugaucaccccuggcaccaacaccagcaaucagguggcagugcuguaccagggcgugaacuguacagaggugccaguggccauucacgccgaucagcugaccccuacuuggcggguguacuccacaggcagcaauguguuucagaccagagccggcugucugaucggagccgagcacgugaacaauagcuacgagugcgacauccccaucggcgcuggcaucugugccagcuaccagacacagacaaacagcccucagcaggcccagucuguggccagccagagcaucauugccuacacaaugucucugggcgccgagaacagcguggccuacuccaacaacucuaucgcuauccccaccaacuucaccaucagcgugaccacagagauccugccuguguccaugaccaagaccagcguggacugcaccauguacaucugcggcgauuccaccgagugcuccaaccugcugcugcaguacggcagcuucugcacccagcugaauagagcccugacagggaucgccguggaacaggacaagaacacccaagagguguucgcccaagugaagcagaucuacaagaccccuccuaucaaggacuucggcggcuucaauuucagccagauucugcccgauccuagcaagcccagcaagcggagcuucaucgaggaccugcuguucaacaaagugacacuggccgacgccggcuucaucaagcaguauggcgauugucugggcgacauugccgccagggaucugauuugcgcccagaaguuuaacggacugacagugcugccuccucugcugaccgaugagaugaucgcccaguacacaucugcccugcuggccggcacaaucacaagcggcuggacauuuggagcuggcgccgcucugcagauccccuuugcuaugcagauggccuaccgguucaacggcaucggagugacccagaaugugcuguacgagaaccagaagcugaucgccaaccaguucaacagcgccaucggcaagauccaggacagccugagcagcacagcaagcgcccugggaaagcugcaggacguggucaaccagaaugcccaggcacugaacacccuggucaagcagcuguccuccaacuucggcgccaucagcucugugcugaacgauauccugagcagacuggacccuccugaggccgaggugcagaucgacagacugaucacaggcagacugcagagccuccagacauacgugacccagcagcugaucagagccgccgagauuagagccucugccaaucuggccgccaccaagaugucugagugugugcugggccagagcaagagaguggacuuuugcggcaagggcuaccaccugaugagcuucccucagucugcaccacacggcgugguguuucugcacgugaccuacgugcccgcucaagagaagaauuucaccaccgcuccagccaucugccacgacggcaaagcccacuuuccuagagaaggcguguucguguccaacggcacccauugguucgugacacagcggaacuucuacgagccccagaucaucaccaccgacaacaccuucgugucuggcaacugcgacgucgugaucggcauugugaacaauaccguguacgacccucugcagcccgagcuggacagcuucaaagaggaacuggacaaguacuuuaagaaccacacaagccccgacguggaccugggcgauaucagcggaaucaaugccagcgucgugaacauccagaaagagaucgaccggcugaacgagguggccaagaaucugaacgagagccugaucgaccugcaagaacuggggaaguacgagcaguacaucaaguggccuugguacaucuggcugggcuuuaucgccggacugauugccaucgugauggucacaaucaugcuguguugcaugaccagcugcuguagcugccugaagggcuguuguagcuguggcagcugcugcaaguucgacgaggacgauucugagcccgugcugaaaggcgugaagcugcacuacaccuga